European Patent Specification EP 4 031 685 B1, published July 10, 2024. Title: IN VITRO FERTILISATION (IVF) EMBRYO VIABILILITY AND QUALITY ASSAY. Applicant: University of Tartu. The sequence listing filed with the application follows.

SEQUENCE LISTING (49 sequences)

SEQ ID NO: 1 - DNA, 21 bp, Artificial Sequence
  qPCR primer
tgatacagaagacttgagatt

SEQ ID NO: 2 - DNA, 21 bp, Artificial Sequence
  qPCR primer
tcacaaagtattcacattacc

SEQ ID NO: 3 - DNA, 21 bp, Artificial Sequence
  qPCR primer
tcaagttcagtgtttggttaa

SEQ ID NO: 4 - DNA, 18 bp, Artificial Sequence
  qPCR primer
ggcagaatcgtgaatagc

SEQ ID NO: 5 - DNA, 22 bp, Artificial Sequence
  qPCR primer
aacaggtcacaatggtggaatg

SEQ ID NO: 6 - DNA, 22 bp, Artificial Sequence
  qPCR primer
tgaagcaactgaagatccacaa

SEQ ID NO: 7 - DNA, 19 bp, Artificial Sequence
  qPCR primer
cgggcattcctgaagctga

SEQ ID NO: 8 - DNA, 20 bp, Artificial Sequence
  qPCR primer
tggagtacgctggatagcct

SEQ ID NO: 9 - DNA, 18 bp, Artificial Sequence
  qPCR primer
gtgcgccgttccgaaagt

SEQ ID NO: 10 - DNA, 21 bp, Artificial Sequence
  qPCR primer
atcatccatggtgagctggcg

SEQ ID NO: 11 - DNA, 18 bp, Artificial Sequence
  qPCR primer
tactgcatcccgctctac

SEQ ID NO: 12 - DNA, 18 bp, Artificial Sequence
  qPCR primer
cgctcatcaagtcgttca

SEQ ID NO: 13 - RNA, 100 nt, Artificial Sequence
  Synthetic RNA spike-in (100 bp from isopenicillin N-CoA synthetase)
uugggcagaaaccgggccccaacggugaccgcaccuacuacugcaucccgcucuaccacggaacggggggcaucgcggccaugaacgacuugaugagcgg

SEQ ID NO: 14 - DNA, 79 bp, Homo sapiens
tgatacagaagacttgagattctggattggagcttgatgccacaattttggatgagaaatttggaggtcctggaatagg

SEQ ID NO: 15 - DNA, 162 bp, Homo sapiens
tcaagttcagtgtttggttaaaatacatactcagtaaatggtagctattattgtcttagtttaagttattgcaagcattaaaattaaatgtttagctacagactcaatccagttttaatgtcattgtgttaataaggcctcttaacattgaagcaacaaaga

SEQ ID NO: 16 - DNA, 82 bp, Homo sapiens
aacaggtcacaatggtggaatgtcgtcagctaaggcaggacctggctatttgcacttcttttgtggatcttcagttgcttca

SEQ ID NO: 17 - RNA, 78 nt, Homo sapiens
ugauacagaagacuugagauucuggauuggagcuugaugccacaauuuuggaugagaaauuuggagguccuggaauag

SEQ ID NO: 18 - RNA, 162 nt, Homo sapiens
ucaaguucaguguuugguuaaaauacauacucaguaaaugguagcuauuauugucuuaguuuaaguuauugcaagcauuaaaauuaaauguuuagcuacagacucaauccaguuuuaaugucauuguguuaauaaggccucuuaacauugaagcaacaaaga

SEQ ID NO: 19 - RNA, 82 nt, Homo sapiens
aacaggucacaaugguggaaugucgucagcuaaggcaggaccuggcuauuugcacuucuuuuguggaucuucaguugcuuca

SEQ ID NO: 20 - DNA, 18 bp, Artificial Sequence
  Primer sequence
gaagcggctgcggttctc

SEQ ID NO: 21 - DNA, 24 bp, Artificial Sequence
  Primer sequence
tgaacgtcgaatcctcctgacaac

SEQ ID NO: 22 - DNA, 20 bp, Artificial Sequence
  Primer sequence
ggatgtggagagttcttgga

SEQ ID NO: 23 - DNA, 18 bp, Artificial Sequence
  Primer sequence
gctggggtcagaaggaag

SEQ ID NO: 24 - DNA, 18 bp, Artificial Sequence
  Primer sequence
cttggagtctctgcggag

SEQ ID NO: 25 - DNA, 20 bp, Artificial Sequence
  Primer sequence
ggctttcttgctgacaactt

SEQ ID NO: 26 - DNA, 22 bp, Artificial Sequence
  Primer sequence
gtgcctgtgaggtatcagtgtc

SEQ ID NO: 27 - DNA, 24 bp, Artificial Sequence
  Primer sequence
gcgtctttgagtagagtccagttg

SEQ ID NO: 28 - DNA, 20 bp, Artificial Sequence
  Primer sequence
gaggatgtgactgtggactt

SEQ ID NO: 29 - DNA, 18 bp, Artificial Sequence
  Primer sequence
gcaggtggctgtagttct

SEQ ID NO: 30 - DNA, 20 bp, Artificial Sequence
  Primer sequence
ggcagcaactggactctact

SEQ ID NO: 31 - DNA, 18 bp, Artificial Sequence
  Primer sequence
tcgaaccccactgagagc

SEQ ID NO: 32 - DNA, 22 bp, Artificial Sequence
  Primer sequence
agttcctaaaccagaggtcatc

SEQ ID NO: 33 - DNA, 18 bp, Artificial Sequence
  Primer sequence
ggcttccccttccaatgt

SEQ ID NO: 34 - DNA, 24 bp, Artificial Sequence
  Primer sequence
gtcatcttcaagttggagcaagga

SEQ ID NO: 35 - DNA, 24 bp, Artificial Sequence
  Primer sequence
atttcccatctgaacagctctgat

SEQ ID NO: 36 - DNA, 22 bp, Artificial Sequence
  Primer sequence
cagtggatgactatggagaaga

SEQ ID NO: 37 - DNA, 21 bp, Artificial Sequence
  Primer sequence
tacagcaggaaggaagatgag

SEQ ID NO: 38 - DNA, 20 bp, Artificial Sequence
  RT qPCR primer
atgtgtcgccccaagaacac

SEQ ID NO: 39 - DNA, 21 bp, Artificial Sequence
  RT qPCR primer
ctcctccgtggaactggattc

SEQ ID NO: 40 - DNA, 25 bp, Artificial Sequence
  RT qPCR primer
ggaagtgaagatatggagtccaaga

SEQ ID NO: 41 - DNA, 21 bp, Artificial Sequence
  RT qPCR primer
agtcgatgaggtcaatgcagg

SEQ ID NO: 42 - DNA, 23 bp, Artificial Sequence
  RT qPCR primer
tcgccataatgaggagggaatta

SEQ ID NO: 43 - DNA, 21 bp, Artificial Sequence
  RT qPCR primer
aaatccagccccaacagagtt

SEQ ID NO: 44 - DNA, 19 bp, Artificial Sequence
  RT qPCR
aaggatggctcgcttcgtg

SEQ ID NO: 45 - DNA, 21 bp, Artificial Sequence
  RT qPCR
atctttggaggacgctggatg

SEQ ID NO: 46 - DNA, 23 bp, Artificial Sequence
  RT qPCR primer
tgtcaagctcatttcctggtacg

SEQ ID NO: 47 - DNA, 21 bp, Artificial Sequence
  RT qPCR primer
gaactcttcctctcgtgctcc

SEQ ID NO: 48 - DNA, 22 bp, Artificial Sequence
  RT qPCR primer
gacactcagcacagtagggttc

SEQ ID NO: 49 - DNA, 20 bp, Artificial Sequence
  RT qPCR primer
atcttgggacacgcagcaag